European Patent Application EP 4 711 474 A1, published March 18, 2026. Title: DNA FRAGMENTS, PRIMER SET AND KIT FOR GENETIC SEX IDENTIFICATION OF ACIPENSER SINENSIS, AND USES. Applicant: CHINESE STURGEON RESEARCH INSTITUTE OF CTG Chinese Sturgeon Research Institute, China Three Gorges Corporation. Application CN. The sequence listing filed with the application follows.

SEQUENCE LISTING (6 sequences)

SEQ ID NO: 1 - DNA, 143 bp, Acipenser sinensis
  source 1..143: mol_type = genomic DNA
taagcgagctgtaagcatcgagctcctggcggctgatttgattttgtttacacttgagaagagccgttccactgtgcatgttgtcaagtcaaagaagtttcactgatccctggtactggcgcatttgttgattcgtcggttcg

SEQ ID NO: 2 - DNA, 122 bp, Acipenser sinensis
  source 1..122: mol_type = genomic DNA
tcaaatcgctccataactgggtgggcccatgagcaaaataggtgggcccaggctcctcaggcccaagcgtggctccgcccctggatacatttgtaaagtgtgttattaggcattccgtagca

SEQ ID NO: 3 - DNA, 19 bp, synthetic construct
  source 1..19: mol_type = other DNA
taagcgagctgtaagcatc

SEQ ID NO: 4 - DNA, 17 bp, synthetic construct
  source 1..17: mol_type = other DNA
cgaaccgacgaatcaac

SEQ ID NO: 5 - DNA, 19 bp, synthetic construct
  source 1..19: mol_type = other DNA
tcaaatcgctccataactg

SEQ ID NO: 6 - DNA, 18 bp, synthetic construct
  source 1..18: mol_type = other DNA
tgctacggaatgcctaat